European Patent Specification EP 3 788 063 B1, published August 9, 2023. Title: GIP derivatives and uses thereof. Applicant: Novo Nordisk A/S. The sequence listing filed with the application follows.

SEQUENCE LISTING (65 sequences)

SEQ ID NO: 1 - protein, 42 aa, HOMO SAPIENS
  misc_feature: hGIP(1-42)
YAEGTFISDYSIAMDKIHQQDFVNWLLAQKGKKNDWKHNITQ

SEQ ID NO: 2 - protein, 31 aa, ARTIFICIAL
  Synthetic polypeptide
  misc_feature: Truncated human GIP(1-31)
YAEGTFISDYSIAMDKIHQQDFVNWLLAQKG

SEQ ID NO: 3 - protein, 31 aa, ARTIFICIAL
  Synthetic polypeptide
  misc_feature: Formula I
  misc_feature (24)..(24): Modifying group attached to epsilon amino group of lysine
YAEGTFISDYSIAMDKIHQQDFVKWLLAQKG

SEQ ID NO: 4 - protein, 31 aa, HOMO SAPIENS
  misc_feature: human GLP-1(7-37)
HAEGTFTSDVSSYLEGQAAKEFIAWLVKGRG

SEQ ID NO: 5 - protein, 29 aa, HOMO SAPIENS
  misc_feature: human glucagon
HSQGTFTSDYSKYLDSRRAQDFVQWLMNT

SEQ ID NO: 6 - protein, 31 aa, ARTIFICIAL
  Synthetic polypeptide
  misc_feature: Compound 1
  misc_feature (2)..(2): Xaa is Aib (alpha-aminoisobutyric acid)
  misc_feature (14)..(14): Xaa is Nle (Norleucine)
  misc_feature (24)..(24): The epsilon amino group of Lys has the following substituent: [(4S)-4-carboxy-4-[[(4S)-4-carboxy-4-[[(4S)-4-carboxy-4-(17-carbo xyheptadecanoylamino)butanoyl]amino]butanoyl]amino]butanoyl]-
YXEGTFISDYSIAXDKIRQQDFVKWLLAQKG

SEQ ID NO: 7 - protein, 31 aa, ARTIFICIAL
  Synthetic polypeptide
  misc_feature: Compound 2
  misc_feature (2)..(2): Xaa is Aib (alpha-aminoisobutyric acid)
  misc_feature (14)..(14): Xaa is Nle (Norleucine)
  misc_feature (24)..(24): The epsilon amino group of Lys has the following substituent: [(4S)-4-carboxy-4-[[(4S)-4-carboxy-4-[[(4S)-4-carboxy-4-(17-carbo xyheptadecanoylamino)butanoyl]amino]butanoyl]amino]butanoyl]-
YXEGTFISDYSIAXDKIHQQDFVKWLLAQKG

SEQ ID NO: 8 - protein, 31 aa, ARTIFICIAL; identical to SEQ ID NO: 6
  Synthetic polypeptide
  misc_feature: Compound 3
  misc_feature (2)..(2): Xaa is Aib (alpha-aminoisobutyric acid)
  misc_feature (14)..(14): Xaa is Nle (Norleucine)
  misc_feature (24)..(24): Epsilon amino group of Lys: [2-[2-[2-[[2-[2-[2-[[(4S)-4-carboxy-4-[[4-[(19-carboxynonadecanoy lamino)methyl]cyclohexanecarbonyl]amino]butanoyl]amino]ethoxy]eth oxy]acetyl]amino]ethoxy] ethoxy]acetyl]-

SEQ ID NO: 9 - protein, 31 aa, ARTIFICIAL; identical to SEQ ID NO: 6
  Synthetic polypeptide
  misc_feature: Compound 4
  misc_feature (2)..(2): Xaa is Aib (alpha-aminoisobutyric acid)
  misc_feature (14)..(14): Xaa is Nle (Norleucine)
  misc_feature (24)..(24): The epsilon amino group of Lys has the following substituent: [(4S)-4-carboxy-4-[[(4S)-4-carboxy-4-[[(4S)-4-carboxy-4-[[4-[(19- carboxynonadecanoylamino)methyl]cyclohexanecarbonyl]amino]butanoy l]amino]butanoyl]amino]butanoyl]-

SEQ ID NO: 10 - protein, 31 aa, ARTIFICIAL
  Synthetic polypeptide
  misc_feature: Compound 5
  misc_feature (1)..(1): Xaa is N-acetyl D-Tyr
  misc_feature (2)..(2): Xaa is Aib (alpha-aminoisobutyric acid)
  misc_feature (14)..(14): Xaa is Nle (Norleucine)
  misc_feature (24)..(24): The epsilon amino group of Lys has the following substituent: [(4S)-4-carboxy-4-[[(4S)-4-carboxy-4-[[(4S)-4-carboxy-4-(17-carbo xyheptadecanoylamino)butanoyl]amino]butanoyl]amino]butanoyl]-
XXEGTFISDYSIAXDKIRQQDFVKWLLAQKG

SEQ ID NO: 11 - protein, 31 aa, ARTIFICIAL; identical to SEQ ID NO: 10
  Synthetic polypeptide
  misc_feature: Compound 6
  misc_feature (1)..(1): Xaa is N-acetyl D-Tyr
  misc_feature (2)..(2): Xaa is Aib (alpha-aminoisobutyric acid)
  misc_feature (14)..(14): Xaa is Nle (Norleucine)
  misc_feature (24)..(24): The epsilon amino group of Lys has the following substituent: [(4S)-4-carboxy-4-[[(4S)-4-carboxy-4-[[(4S)-4-carboxy-4-[[4-[(19- carboxynonadecanoylamino)methyl]cyclohexanecarbonyl]amino]butanoy l] amino]butanoyl]amino]butanoyl]-

SEQ ID NO: 12 - protein, 31 aa, ARTIFICIAL
  Synthetic polypeptide
  misc_feature: Compound 7
  misc_feature (1)..(1): Xaa is N-acetyl D-Tyr
  misc_feature (14)..(14): Xaa is Nle (Norleucine)
  misc_feature (24)..(24): The epsilon amino group of Lys has the following substituent: [(4S)-4-carboxy-4-[[(4S)-4-carboxy-4-[[(4S)-4-carboxy-4-(17-carbo xyheptadecanoylamino)butanoyl]amino]butanoyl]amino]butanoyl]-
XAEGTFISDYSIAXDKIRQQDFVKWLLAQKG

SEQ ID NO: 13 - protein, 31 aa, ARTIFICIAL; identical to SEQ ID NO: 12
  Synthetic polypeptide
  misc_feature: Compound 8
  misc_feature (1)..(1): Xaa is N-acetyl D-Tyr
  misc_feature (14)..(14): Xaa is Nle (Norleucine)
  misc_feature (24)..(24): The epsilon amino group of Lys has the following substituent: [(4S)-4-carboxy-4-[[(4S)-4-carboxy-4-[[(4S)-4-carboxy-4-[[4-[(19- carboxynonadecanoylamino)methyl]cyclohexanecarbonyl]amino]-butano yl]amino]butanoyl]amino]butanoyl]-

SEQ ID NO: 14 - protein, 31 aa, ARTIFICIAL
  Synthetic polypeptide
  misc_feature: Compound 9
  misc_feature (2)..(2): Xaa is Aib (alpha-aminoisobutyric acid)
  misc_feature (14)..(14): Xaa is Nle (Norleucine)
  misc_feature (24)..(24): The epsilon amino group of Lys has the following substituent: [(4S)-4-carboxy-4-[[(4S)-4-carboxy-4-[[(4S)-4-carboxy-4-(17-carbo xyheptadecanoylamino)butanoyl]amino]butanoyl]amino]butanoyl]-
YXEGTFISDYSIAXDKIRQEDFVKWLLAQKG

SEQ ID NO: 15 - protein, 31 aa, ARTIFICIAL; identical to SEQ ID NO: 14
  Synthetic polypeptide
  misc_feature: Compound 10
  misc_feature (2)..(2): Xaa is Aib (alpha-aminoisobutyric acid)
  misc_feature (14)..(14): Xaa is Nle (Norleucine)
  misc_feature (24)..(24): The epsilon amino group of Lys has the following substituent: [(4S)-4-carboxy-4-[[(4S)-4-carboxy-4-[[(4S)-4-carboxy-4-[[4-[(19- carboxynonadecanoylamino)methyl]cyclohexanecarbonyl]amino]butanoy l]amino]-butanoyl]amino]butanoyl]-

SEQ ID NO: 16 - protein, 31 aa, ARTIFICIAL
  Synthetic polypeptide
  misc_feature: Compound 11
  misc_feature (2)..(2): Xaa is Aib (alpha-aminoisobutyric acid)
  misc_feature (14)..(14): Xaa is Nle (Norleucine)
  misc_feature (20)..(20): Xaa is Aib (alpha-aminoisobutyric acid)
  misc_feature (24)..(24): The epsilon amino group of Lys has the following substituent: [(4S)-4-carboxy-4-[[(4S)-4-carboxy-4-[[(4S)-4-carboxy-4-(17-carbo xyheptadecanoylamino)butanoyl]amino]butanoyl]amino]butanoyl]-
YXEGTFISDYSIAXDKIRQXDFVKWLLAQKG

SEQ ID NO: 17 - protein, 31 aa, ARTIFICIAL; identical to SEQ ID NO: 16
  Synthetic polypeptide
  misc_feature: Compound 12
  misc_feature (2)..(2): Xaa is Aib (alpha-aminoisobutyric acid)
  misc_feature (14)..(14): Xaa is Nle (Norleucine)
  misc_feature (20)..(20): Xaa is Aib (alpha-aminoisobutyric acid)
  misc_feature (24)..(24): The epsilon amino group of Lys has the following substituent: [(4S)-4-carboxy-4-[[(4S)-4-carboxy-4-[[(4S)-4-carboxy-4-[[4-[(19- carboxynonadecanoylamino)methyl]cyclohexanecarbonyl]amino]butanoy l]amino]-butanoyl]amino]butanoyl]-

SEQ ID NO: 18 - protein, 31 aa, ARTIFICIAL
  Synthetic polypeptide
  misc_feature: Compound 13
  misc_feature (2)..(2): Xaa is Aib (alpha-aminoisobutyric acid)
  misc_feature (14)..(14): Xaa is Nle (Norleucine)
  misc_feature (24)..(24): The epsilon amino group of Lys has the following substituent: [(4S)-4-carboxy-4-[[(4S)-4-carboxy-4-[[(4S)-4-carboxy-4-(17-carbo xyheptadecanoylamino)butanoyl]amino]butanoyl]amino]butanoyl]-
YXEGTFISDYSIAXDAIRQQDFVKWLLAQKG

SEQ ID NO: 19 - protein, 31 aa, ARTIFICIAL; identical to SEQ ID NO: 18
  Synthetic polypeptide
  misc_feature: Compound 14
  misc_feature (2)..(2): Xaa is Aib (alpha-aminoisobutyric acid)
  misc_feature (14)..(14): Xaa is Nle (Norleucine)
  misc_feature (24)..(24): The epsilon amino group of Lys has the following substituent: [(4S)-4-carboxy-4-[[(4S)-4-carboxy-4-[[(4S)-4-carboxy-4-[[4-[(19- carboxynonadecanoylamino)methyl]cyclohexanecarbonyl]amino]butanoy l]amino]-butanoyl]amino]butanoyl]-

SEQ ID NO: 20 - protein, 31 aa, ARTIFICIAL; identical to SEQ ID NO: 12
  Synthetic polypeptide
  misc_feature: Compound 15
  misc_feature (1)..(1): Xaa is N-acetyl D-Tyr
  misc_feature (14)..(14): Xaa is Nle (Norleucine)
  misc_feature (24)..(24): The epsilon amino group of Lys has the following substituent: [2-[2-[2-[[2-[2-[2-[[(4S)-4-carboxy-4-(17-carboxyheptadecanoylami no)butanoyl]amino]ethoxy]ethoxy]acetyl]amino]ethoxy]ethoxy]acetyl ]-

SEQ ID NO: 21 - protein, 31 aa, ARTIFICIAL
  Synthetic polypeptide
  misc_feature: Compound 16
  misc_feature (1)..(1): Xaa is N-acetyl D-Tyr
  misc_feature (14)..(14): Xaa is Nle (Norleucine)
  misc_feature (24)..(24): The epsilon amino group of Lys has the following substituent: [2-[2-[2-[[2-[2-[2-[[(4S)-4-carboxy-4-(17-carboxy-heptadecanoylam ino)butanoyl]amino]ethoxy]ethoxy]acetyl]amino]ethoxy]ethoxy]acety l]-
XAEGTFISDYSIAXDKIRQEDFVKWLLAQKG

SEQ ID NO: 22 - protein, 31 aa, ARTIFICIAL; identical to SEQ ID NO: 12
  Synthetic polypeptide
  misc_feature: Compound 17
  misc_feature (1)..(1): Xaa is N-acetyl D-Tyr
  misc_feature (14)..(14): Xaa is Nle (Norleucine)
  misc_feature (24)..(24): Epsilon NH2 group of Lys has:[2-[2-[2-[[2-[2-[2-[[(4S)- 4-carboxy-4-[[(4S)-4-carboxy-4-[[(4S)-4-carboxy-4-(17-carboxyhept adecanoylamino)butanoyl]amino]butanoyl]amino]-butanoyl]amino]etho xy]ethoxy]acetyl]amino]ethoxy]ethoxy]acetyl]-

SEQ ID NO: 23 - protein, 31 aa, ARTIFICIAL
  Synthetic polypeptide
  misc_feature: Compound 18
  misc_feature (1)..(1): N-terminal Acetyl
  misc_feature (14)..(14): Xaa is Nle (Norleucine)
  misc_feature (24)..(24): The epsilon amino group of Lys has the following substituent: [(4S)-4-carboxy-4-[[(4S)-4-carboxy-4-[[(4S)-4-carboxy-4-(17-carbo xyheptadecanoylamino)butanoyl]amino]butanoyl]amino]butanoyl]-
YAEGTFISDYSIAXDKIRQQDFVKWLLAQKG

SEQ ID NO: 24 - protein, 31 aa, ARTIFICIAL
  Synthetic polypeptide
  misc_feature: Compound 19
  misc_feature (1)..(1): Xaa is N-acetyl D-Tyr
  misc_feature (24)..(24): The epsilon amino group of Lys has the following substituent: [2-[2-[2-[[2-[2-[2-[[(4S)-4-carboxy-4-(17-carboxyheptadecanoylami no)butanoyl]amino]ethoxy]ethoxy]acetyl]amino]ethoxy]ethoxy]acetyl ]-
XAEGTFISDYSIADDKIRQEDFVKWLLAQKG

SEQ ID NO: 25 - protein, 31 aa, ARTIFICIAL
  Synthetic polypeptide
  misc_feature: Compound 20
  misc_feature (2)..(2): Xaa is Aib (alpha-aminoisobutyric acid)
  misc_feature (14)..(14): Xaa is Nle (Norleucine)
  misc_feature (24)..(24): The epsilon amino group of Lys has the following substituent: [(4S)-4-carboxy-4-[[(4S)-4-carboxy-4-[[(4S)-4-carboxy-4-[[(4S)-4- carboxy-4-(17-carboxyheptadecanoylamino)butanoyl]amino]butanoyl]a mino]butanoyl]-amino]butanoyl]-
YXEGTFISDYSIAXDKIHQEDFVKWLLAQKG

SEQ ID NO: 26 - protein, 31 aa, ARTIFICIAL; identical to SEQ ID NO: 25
  Synthetic polypeptide
  misc_feature: Compound 21
  misc_feature (2)..(2): Xaa is Aib (alpha-aminoisobutyric acid)
  misc_feature (14)..(14): Xaa is Nle (Norleucine)
  misc_feature (24)..(24): Epsilon amino group of Lys has:[(4S)-4-carboxy-4-[[(4S)- 4-carboxy-4-[[(4S)-4-carboxy-4-[[(4S)-4-carboxy-4-[[4-[(19-carbox ynonadecanoylamino)methyl]cyclohexanecarbonyl]-amino]butanoyl]-am ino]butanoyl]amino]butanoyl]amino]butanoyl]-

SEQ ID NO: 27 - protein, 31 aa, ARTIFICIAL
  Synthetic polypeptide
  misc_feature: Compound 22
  misc_feature (1)..(1): Xaa is N-acetyl D-Tyr
  misc_feature (14)..(14): Xaa is Nle (Norleucine)
  misc_feature (24)..(24): The epsilon amino group of Lys has the following substituent: [(4S)-4-carboxy-4-[[(4S)-4-carboxy-4-[[(4S)-4-carboxy-4-[[4-[(19- carboxynonadecanoylamino)methyl]cyclohexanecarbonyl]amino]butanoy l]-amino]butanoyl]amino]butanoyl]-
XAEGTFISDYSIAXDKIHQEDFVKWLLAQKG

SEQ ID NO: 28 - protein, 31 aa, ARTIFICIAL; identical to SEQ ID NO: 21
  Synthetic polypeptide
  misc_feature: Compound 23
  misc_feature (1)..(1): Xaa is N-acetyl D-Tyr
  misc_feature (14)..(14): Xaa is Nle (Norleucine)
  misc_feature (24)..(24): The epsilon amino group of Lys has the following substituent: [(4S)-4-carboxy-4-[[(4S)-4-carboxy-4-[[(4S)-4-carboxy-4-[[4-[(19- carboxynonadecanoylamino)methyl]cyclohexanecarbonyl]amino]butanoy l]-amino]butanoyl]amino]butanoyl]-

SEQ ID NO: 29 - protein, 31 aa, ARTIFICIAL
  Synthetic polypeptide
  misc_feature: Compound 24
  misc_feature (1)..(1): Xaa is N-acetyl D-Tyr
  misc_feature (14)..(14): Xaa is Nle (Norleucine)
  misc_feature (20)..(20): Xaa is Aib (alpha-aminoisobutyric acid)
  misc_feature (24)..(24): The epsilon amino group of Lys has the following substituent: [(4S)-4-carboxy-4-[[(4S)-4-carboxy-4-[[(4S)-4-carboxy-4-[[4-[(19- carboxynonadecanoylamino)methyl]cyclohexanecarbonyl]amino]butanoy l]-amino]butanoyl]amino]butanoyl]-
XAEGTFISDYSIAXDKIHQXDFVKWLLAQKG

SEQ ID NO: 30 - protein, 31 aa, ARTIFICIAL
  Synthetic polypeptide
  misc_feature: Compound 25
  misc_feature (1)..(1): Xaa is N-acetyl D-Tyr
  misc_feature (14)..(14): Xaa is Nle (Norleucine)
  misc_feature (20)..(20): Xaa is Aib (alpha-aminoisobutyric acid)
  misc_feature (24)..(24): The epsilon amino group of Lys has the following substituent: [(4S)-4-carboxy-4-[[(4S)-4-carboxy-4-[[(4S)-4-carboxy-4-[[4-[(19- carboxynonadecanoylamino)methyl]cyclohexanecarbonyl]amino]butanoy l]-amino]butanoyl]amino]butanoyl]-
XAEGTFISDYSIAXDKIRQXDFVKWLLAQKG

SEQ ID NO: 31 - protein, 31 aa, ARTIFICIAL
  Synthetic polypeptide
  misc_feature: Compound 26
  misc_feature (2)..(2): Xaa is Aib (alpha-aminoisobutyric acid)
  misc_feature (14)..(14): Xaa is Nle (Norleucine)
  misc_feature (24)..(24): The epsilon amino group of Lys has the following substituent: [(4S)-4-carboxy-4-[[(4S)-4-carboxy-4-[[(4S)-4-carboxy-4-[[4-[(19- carboxynonadecanoylamino)methyl]cyclohexanecarbonyl]amino]butanoy l]amino]-butanoyl]amino]butanoyl]-
  misc_feature (31)..(31): C-terminal amidation
YXEGTFISDYSIAXDKIRQQDFVKWLLAQKP

SEQ ID NO: 32 - protein, 31 aa, ARTIFICIAL
  Synthetic polypeptide
  misc_feature: Compound 27
  misc_feature (2)..(2): Xaa is Aib (alpha-aminoisobutyric acid)
  misc_feature (14)..(14): Xaa is Nle (Norleucine)
  misc_feature (24)..(24): The epsilon amino group of Lys has the following substituent: [(4S)-4-carboxy-4-[[(4S)-4-carboxy-4-[[(4S)-4-carboxy-4-[[4-[(19- carboxynonadecanoylamino)methyl]cyclohexanecarbonyl]amino]butanoy l]amino]-butanoyl]amino]butanoyl]-
  misc_feature (31)..(31): C-terminal amidation
YXEGTFISDYSIAXDKIHQQDFVKWLLAQKP

SEQ ID NO: 33 - protein, 31 aa, ARTIFICIAL
  Synthetic polypeptide
  misc_feature: Compound 28
  misc_feature (1)..(1): Xaa is N-acetyl D-Tyr
  misc_feature (14)..(14): Xaa is Nle (Norleucine)
  misc_feature (24)..(24): The epsilon amino group of Lys has the following substituent: [(4S)-4-carboxy-4-[[(4S)-4-carboxy-4-[[(4S)-4-carboxy-4-[[4-[(19- carboxynonadecanoylamino)methyl]cyclohexanecarbonyl]amino]butanoy l]-amino]butanoyl]amino]butanoyl]-
  misc_feature (31)..(31): C-terminal amidation
XAEGTFISDYSIAXDKIRQQDFVKWLLAQKP

SEQ ID NO: 34 - protein, 31 aa, ARTIFICIAL
  Synthetic polypeptide
  misc_feature: Compound 29
  misc_feature (1)..(1): Xaa is N-acetyl D-Tyr
  misc_feature (14)..(14): Xaa is Nle (Norleucine)
  misc_feature (24)..(24): The epsilon amino group of Lys has the following substituent: [(4S)-4-carboxy-4-[[(4S)-4-carboxy-4-[[(4S)-4-carboxy-4-[[4-[(19- carboxynonadecanoylamino)methyl]cyclohexanecarbonyl]amino]butanoy l]-amino]butanoyl]amino]butanoyl]-
  misc_feature (31)..(31): C-terminal amidation
XAEGTFISDYSIAXDKIHQQDFVKWLLAQKP

SEQ ID NO: 35 - protein, 31 aa, ARTIFICIAL; identical to SEQ ID NO: 12
  Synthetic polypeptide
  misc_feature: Compound 30
  misc_feature (1)..(1): Xaa is N-acetyl D-Tyr
  misc_feature (14)..(14): Xaa is Nle (Norleucine)
  misc_feature (24)..(24): Epsilon amino group of Lys has:[(4S)-4-carboxy-4- [[(4S)-4-carboxy-4-[[(4S)-4-carboxy-4-[[(4S)-4-carboxy-4-[[4-[(19 -carboxynonadecanoylamino)methyl]cyclohexanecarbonyl]-amino]butan oyl]amino]butanoyl]amino]butanoyl]amino]butanoyl]-

SEQ ID NO: 36 - protein, 31 aa, ARTIFICIAL
  Synthetic polypeptide
  misc_feature: Compound 31
  misc_feature (1)..(1): Xaa is N-acetyl D-Tyr
  misc_feature (2)..(2): Xaa is Aib (alpha-aminoisobutyric acid)
  misc_feature (14)..(14): Xaa is Nle (Norleucine)
  misc_feature (24)..(24): The epsilon amino group of Lys has:[(4S)-4-carboxy-4- [[(4S)-4-carboxy-4-[[(4S)-4-carboxy-4-[[(4S)-4-carboxy-4-[[4-[(19 -carboxynonadecanoylamino)methyl]cyclohexanecarbonyl]-amino]butan oyl]amino]butanoyl]amino]butanoyl]amino]butanoyl]-
  misc_feature (31)..(31): C-terminal amidation
XXEGTFISDYSIAXDKIRQQDFVKWLLAQKP

SEQ ID NO: 37 - protein, 31 aa, ARTIFICIAL
  Synthetic polypeptide
  misc_feature: Compound 32
  misc_feature (1)..(1): Xaa is N-acetyl D-Tyr
  misc_feature (2)..(2): Xaa is Aib (alpha-aminoisobutyric acid)
  misc_feature (14)..(14): Xaa is Nle (Norleucine)
  misc_feature (24)..(24): The epsilon amino group of Lys has the following substituent: [(4S)-4-carboxy-4-[[(4S)-4-carboxy-4-[[(4S)-4-carboxy-4-[[4-[(19- carboxynonadecanoylamino)methyl]cyclohexanecarbonyl]amino]butanoy l]-amino]butanoyl]amino]butanoyl]-
  misc_feature (31)..(31): C-terminal amidation
XXEGTFISDYSIAXDKIHQQDFVKWLLAQKP

SEQ ID NO: 38 - protein, 42 aa, ARTIFICIAL
  Synthetic polypeptide
  misc_feature: Compound 33
  misc_feature (2)..(2): Xaa is Aib (alpha-aminoisobutyric acid)
  misc_feature (14)..(14): Xaa is Nle (Norleucine)
  misc_feature (24)..(24): The epsilon amino group of Lys has the following substituent: [(4S)-4-carboxy-4-[[(4S)-4-carboxy-4-[[(4S)-4-carboxy-4-(17-carbo xyheptadecanoylamino)butanoyl]amino]butanoyl]amino]butanoyl]-
YXEGTFISDYSIAXDKIHQQDFVKWLLAQKGKENDWKHNITQ

SEQ ID NO: 39 - protein, 42 aa, ARTIFICIAL
  Synthetic polypeptide
  misc_feature: Compound 34
  misc_feature (2)..(2): Xaa is Aib (alpha-aminoisobutyric acid)
  misc_feature (14)..(14): Xaa is Nle (Norleucine)
  misc_feature (24)..(24): [(4S)-4-carboxy-4-[[(4S)-4-carboxy-4-[[(4S)-4-carboxy-4-(17-carbo xyheptadecanoylamino)butanoyl]amino]butanoyl]amino]butanoyl]-
YXEGTFISDYSIAXDKIRQQDFVKWLLAQKGKENDWKHNITQ

SEQ ID NO: 40 - protein, 42 aa, ARTIFICIAL
  Synthetic polypeptide
  misc_feature: Compound 35
  misc_feature (2)..(2): Xaa is Aib (alpha-aminoisobutyric acid)
  misc_feature (14)..(14): Xaa is Nle (Norleucine)
  misc_feature (24)..(24): The epsilon amino group of Lys has the following substituent: [2-[2-[2-[[2-[2-[2-[[(4S)-4-carboxy-4-(17-carboxyheptadecanoylami no)butanoyl]amino]ethoxy]ethoxy]acetyl]amino]ethoxy]ethoxy]acetyl ]-
YXEGTFISDYSIAXDKIHQQDFVKWLLAQKGKEEDWKHNITQ

SEQ ID NO: 41 - protein, 42 aa, ARTIFICIAL
  Synthetic polypeptide
  misc_feature: Compound 36
  misc_feature (2)..(2): Xaa is Aib (alpha-aminoisobutyric acid)
  misc_feature (14)..(14): Xaa is Nle (Norleucine)
  misc_feature (24)..(24): The epsilon amino group of Lys has the following substituent: [2-[2-[2-[[2-[2-[2-[[(4S)-4-carboxy-4-(17-carboxyheptadecanoylami no)butanoyl]amino]ethoxy]ethoxy]acetyl]amino]ethoxy]ethoxy]acetyl ]-
YXEGTFISDYSIAXDKIHQQDFVKWLLAQKGKEDDWKHNITQ

SEQ ID NO: 42 - protein, 42 aa, ARTIFICIAL
  Synthetic polypeptide
  misc_feature: Compound 37
  misc_feature (2)..(2): Xaa is Aib (alpha-aminoisobutyric acid)
  misc_feature (14)..(14): Xaa is Nle (Norleucine)
  misc_feature (24)..(24): The epsilon amino group of Lys has the following substituent: [2-[2-[2-[[2-[2-[2-[[(4S)-4-carboxy-4-(17-carboxyheptadecanoylami no)butanoyl]amino]ethoxy]ethoxy]acetyl]amino]ethoxy]ethoxy]acetyl ]-
YXEGTFISDYSIAXDKIRQQDFVKWLLAQKGKEEDWKHNITQ

SEQ ID NO: 43 - protein, 42 aa, ARTIFICIAL; identical to SEQ ID NO: 40
  Synthetic polypeptide
  misc_feature: Compound 38
  misc_feature (2)..(2): Xaa is Aib (alpha-aminoisobutyric acid)
  misc_feature (14)..(14): Xaa is Nle (Norleucine)
  misc_feature (24)..(24): The epsilon amino group of Lys has the following substituent: [(4S)-4-carboxy-4-[[(4S)-4-carboxy-4-[[(4S)-4-carboxy-4-(17-carbo xyheptadecanoylamino)butanoyl]amino]butanoyl]amino]butanoyl]-

SEQ ID NO: 44 - protein, 42 aa, ARTIFICIAL; identical to SEQ ID NO: 41
  Synthetic polypeptide
  misc_feature: Compound 39
  misc_feature (2)..(2): Xaa is Aib (alpha-aminoisobutyric acid)
  misc_feature (14)..(14): Xaa is Nle (Norleucine)
  misc_feature (24)..(24): The epsilon amino group of Lys has the following substituent: [(4S)-4-carboxy-4-[[(4S)-4-carboxy-4-[[(4S)-4-carboxy-4-(17-carbo xyheptadecanoylamino)butanoyl]amino]butanoyl]amino]butanoyl]-

SEQ ID NO: 45 - protein, 42 aa, ARTIFICIAL; identical to SEQ ID NO: 42
  Synthetic polypeptide
  misc_feature: Compound 40
  misc_feature (2)..(2): Xaa is Aib (alpha-aminoisobutyric acid)
  misc_feature (14)..(14): Xaa is Nle (Norleucine)
  misc_feature (24)..(24): The epsilon amino group of Lys has the following substituent: [(4S)-4-carboxy-4-[[(4S)-4-carboxy-4-[[(4S)-4-carboxy-4-(17-carbo xyheptadecanoylamino)butanoyl]amino]butanoyl]amino]butanoyl]-

SEQ ID NO: 46 - protein, 42 aa, ARTIFICIAL; identical to SEQ ID NO: 42
  Synthetic polypeptide
  misc_feature: Compound 41
  misc_feature (2)..(2): Xaa is Aib (alpha-aminoisobutyric acid)
  misc_feature (14)..(14): Xaa is Nle (Norleucine)
  misc_feature (24)..(24): The epsilon amino group of Lys has the following substituent: [2-[2-[2-[[2-[2-[2-[[(4S)-4-carboxy-4-[[4-[(19-carboxynonadecanoy l-amino)methyl]cyclohexanecarbonyl]amino]butanoyl]amino]ethoxy]et hoxy]acetyl]amino]ethoxy]ethoxy]acetyl]-

SEQ ID NO: 47 - protein, 42 aa, ARTIFICIAL; identical to SEQ ID NO: 42
  Synthetic polypeptide
  misc_feature: Compound 42
  misc_feature (2)..(2): Xaa is Aib (alpha-aminoisobutyric acid)
  misc_feature (14)..(14): Xaa is Nle (Norleucine)
  misc_feature (24)..(24): The epsilon amino group of Lys has the following substituent: [(4S)-4-carboxy-4-[[(4S)-4-carboxy-4-[[(4S)-4-carboxy-4-[[4-[(19- carboxynonadecanoylamino)methyl]cyclohexanecarbonyl]amino]butanoy l]amino]butanoyl]amino]butanoyl]-

SEQ ID NO: 48 - protein, 31 aa, ARTIFICIAL
  Synthetic polypeptide
  misc_feature: Formula II
  misc_feature (1)..(1): Xaa is any amino acid
  misc_feature (2)..(2): Xaa is any amino acid
  misc_feature (14)..(14): Xaa is any amino acid
  misc_feature (16)..(16): Xaa is any amino acid
  misc_feature (18)..(18): Xaa is any amino acid
  misc_feature (20)..(20): Xaa is any amino acid
  misc_feature (24)..(24): Modifying group attached to epsilon amino group of lysine
  misc_feature (31)..(31): Xaa is any amino acid
XXEGTFISDYSIAXDXIXQXDFVKWLLAQKX

SEQ ID NO: 49 - protein, 31 aa, ARTIFICIAL; identical to SEQ ID NO: 48
  Synthetic polypeptide
  misc_feature (1)..(1): Xaa is Tyr or d-Tyr
  misc_feature (2)..(2): Xaa is Ala, d-Ala, or Aib (alpha-aminoisobutyric acid)
  misc_feature (14)..(14): Xaa is Leu, Met, Asp or Nle (norleucine)
  misc_feature (16)..(16): Xaa is Lys or Ala
  misc_feature (18)..(18): Xaa is Arg or His
  misc_feature (20)..(20): Xaa is Gln, Glu, or Aib (alpha-aminoisobutyric acid)
  misc_feature (24)..(24): Modifying group attached to epsilon amino group of lysine
  misc_feature (31)..(31): Xaa is Gly or Pro

SEQ ID NO: 50 - protein, 31 aa, ARTIFICIAL; identical to SEQ ID NO: 48
  Synthetic polypeptide
  misc_feature (1)..(1): Xaa is Tyr or d-Tyr
  misc_feature (2)..(2): Xaa is Ala or Aib (alpha-aminoisobutyric acid)
  misc_feature (14)..(14): Xaa is Nle (norleucine)
  misc_feature (16)..(16): Xaa is Lys or Ala
  misc_feature (18)..(18): Xaa is His or Arg
  misc_feature (20)..(20): Xaa is Gln, Glu, or Aib (alpha-aminoisobutyric acid)
  misc_feature (24)..(24): Modifying group attached to epsilon amino group of lysine
  misc_feature (31)..(31): Xaa is Gly or Pro

SEQ ID NO: 51 - protein, 11 aa, ARTIFICIAL
  Synthetic polypeptide
  misc_feature: Formula III
  misc_feature (2)..(2): Xaa is Lys or Glu
  misc_feature (3)..(3): Xaa is Asn, Glu, or Asp
KXXDWKHNITQ

SEQ ID NO: 52 - protein, 29 aa, ARTIFICIAL
  Synthetic polypeptide
  Misc_feature: Embodiment 109
  Misc_feature (2)..(2): Xaa is Acb (1-aminocyclobutanecarboxylic acid)
  Misc_feature (28)..(28): Epsilon Lys:[(4S)-4-carboxy-4-[[(4S)-4-carboxy-4-[[2-[2-[2-[[2- [2-[2-[[(4S)-4-carboxy-4-[[(4S)-4-carboxy-4-(17-carboxy heptadecanoylamino)butanoyl]amino]butanoyl]amino]ethoxy]ethoxy] acetyl]amino]ethoxy]ethoxy]acetyl]amino]butanoyl]amino]butanoyl-
  Misc_feature (29)..(29): C-terminal amidation
HXQGTFTSDLSKYLDLRRARDFVQWLLKT

SEQ ID NO: 53 - protein, 29 aa, ARTIFICIAL
  Synthetic polypeptide
  Misc_feature: Embodiment 110
  Misc_feature (2)..(2): Xaa is Aib (alpha-aminoisobutyric acid)
  Misc_feature (28)..(28): Epsilon amino Lys: [(4S)-4-carboxy-4-[[(4S)-4-carboxy-4-[[(2S)-2-[[(2S)-4-carboxy-2- [[(2S)-2-[[(4S)-4-carboxy-4-[[(4S)-4-carboxy-4-(17-carboxyheptade canoylamino)butanoyl]amino]butanoyl]amino]
  Misc_feature (28)..(28): -3-hydroxypropanoyl]amino]butanoyl]amino]-3-hydroxypropanoyl]amin o]butanoyl]amino]butanoyl-
  Misc_feature (29)..(29): C-terminal amidation
HXQGTFTSDLSKYLESKRAREFVQWLLKT

SEQ ID NO: 54 - protein, 29 aa, ARTIFICIAL
  Synthetic polypeptide
  Misc_feature: Embodiment 111
  Misc_feature (2)..(2): Xaa is Acb (1-aminocyclobutanecarboxylic acid)
  Misc_feature (28)..(28): Epsilon amino of Lys: [(4S)-4-carboxy-4-[[(4S)-4- carboxy-4-[[2-[2-[2-[[2-[2-[2-[[(4S)-4-carboxy-4-(17-carboxyhepta decanoylamino)butanoyl]amino]ethoxy]ethoxy]acetyl]amino]ethoxy]et hoxy]acetyl]amino]butanoyl]amino]butanoyl]-
  Misc_feature (29)..(29): C-terminal amidation
HXQGTFTSDLSKYLESRRAREFVQWLLKT

SEQ ID NO: 55 - protein, 29 aa, ARTIFICIAL
  Synthetic polypeptide
  Misc_feature: Embodiment 112
  Misc_feature (2)..(2): Xaa is Acb (1-aminocyclobutanecarboxylic acid)
  Misc_feature (28)..(28): [(4S)-4-carboxy-4-[[(4S)-4-carboxy-4-[[2-[2-[2-[[2-[2-[2-[[(4S)-4 -carboxy-4-[[(4S)-4-carboxy-4-(17-carboxyheptadecanoylamino)butan oyl]amino]butanoyl]amino]ethoxy]ethoxy]acetyl]amino]ethoxy]ethoxy ]acetyl]amino]butanoyl]amino]butanoyl]-
  Misc_feature (29)..(29): C-terminal amidation
HXQGTFTSDLSKYLDLKRAREFVQWLLKT

SEQ ID NO: 56 - protein, 29 aa, ARTIFICIAL
  Synthetic polypeptide
  Misc_feature: Embodiment 113
  Misc_feature (2)..(2): Xaa is Aib (alpha-aminoisobutyric acid)
  Misc_feature (28)..(28): [2-[2-[2-[[2-[2-[2-[[(4S)-4-carboxy-4-[[(4S)-4-carboxy-4-[[(4S)-4 -carboxy-4-(17-carboxyheptadecanoylamino)butanoyl]amino]butanoyl] amino]butanoyl]amino]ethoxy]ethoxy]acetyl]amino]ethoxy]ethoxy]ace tyl]-
  Misc_feature (29)..(29): C-terminal amidation
HXQGTFTSDLSKYLDARRARDFVQWLLKT

SEQ ID NO: 57 - protein, 31 aa, ARTIFICIAL
  Synthetic polypeptide
  MISC_FEATURE: Semaglutide
  MISC_FEATURE (2)..(2): Xaa is Aib (alpha-aminoisobutyric acid)
  MISC_FEATURE (20)..(20): The epsilon amino group of Lys has the following substituent:[2-(2-[2-(2-[2-(2-[4-(17-Carboxyheptadecanoylamino)-4 (S)-carboxybutyrylamino]ethoxy)ethoxy]acetylamino)ethoxy]ethoxy)a cetyl]-
HXEGTFTSDVSSYLEGQAAKEFIAWLVRGRG

SEQ ID NO: 58 - protein, 31 aa, ARTIFICIAL; identical to SEQ ID NO: 57
  Synthetic polypeptide
  MISC_FEATURE: Semaglutide-like molecule
  MISC_FEATURE (2)..(2): Xaa is Aib (alpha-aminoisobutyric acid)
  MISC_FEATURE (20)..(20): The epsilon amino group of Lys has the following substituent: [2-(2-[2-(2-[2-(2-[4-(17-Carboxyheptadecanoylamino)-4(R)-carboxyb utyrylamino]ethoxy)ethoxy]acetylamino)ethoxy]ethoxy)acetyl]-

SEQ ID NO: 59 - protein, 31 aa, ARTIFICIAL; identical to SEQ ID NO: 30
  Synthetic polypeptide
  MISC_FEATURE: Compound 43
  MISC_FEATURE (1)..(1): Xaa is N-acetyl D-Tyr
  MISC_FEATURE (14)..(14): Xaa is Nle (Norleucine)
  MISC_FEATURE (20)..(20): Xaa is Aib (alpha-aminoisobutyric acid)
  MISC_FEATURE (24)..(24): The epsilon amino group of Lys has the following substituent: [2-[2-[2-[[2-[2-[2-[[4-[(19-carboxynonadecanoylamino)methyl]cyclo hexanecarbonyl]amino]ethoxy]ethoxy]acetyl]amino]ethoxy]ethoxy]ace tyl]-

SEQ ID NO: 60 - protein, 31 aa, ARTIFICIAL; identical to SEQ ID NO: 36
  Synthetic polypeptide
  MISC_FEATURE: Compound 44
  MISC_FEATURE (1)..(1): Xaa is N-acetyl D-Tyr
  MISC_FEATURE (2)..(2): Xaa is Aib (alpha-aminoisobutyric acid)
  MISC_FEATURE (14)..(14): Xaa is Nle (Norleucine)
  MISC_FEATURE (24)..(24): The epsilon amino group of Lys has the following substituent: [2-[2-[2-[[2-[2-[2-[[4-[(19-carboxynonadecanoylamino)methyl]cyclo hexanecarbonyl]amino]ethoxy]ethoxy]acetyl]amino]ethoxy]ethoxy]ace tyl]-
  MISC_FEATURE (31)..(31): C-terminal amidation

SEQ ID NO: 61 - protein, 42 aa, ARTIFICIAL
  Synthetic polypeptide
  MISC_FEATURE: Compound 45
  MISC_FEATURE (2)..(2): Xaa is Aib (alpha-aminoisobutyric acid)
  MISC_FEATURE (24)..(24): The epsilon amino group of Lys has the following substituent:[2-[2-[2-[[2-[2-[2-[[(4S)-4-carboxy-4-(17-carboxyhept adecanoylamino)butanoyl]amino]ethoxy]ethoxy]acetyl]amino]ethoxy]e thoxy]acetyl]-
YXEGTFISDYSIALDKIHQQDFVKWLLAQKGKKNDWKHNITQ

SEQ ID NO: 62 - protein, 31 aa, ARTIFICIAL; identical to SEQ ID NO: 36
  Synthetic polypeptide
  MISC_FEATURE: Compound 46
  MISC_FEATURE (1)..(1): Xaa is N-acetyl D-Tyr
  MISC_FEATURE (2)..(2): Xaa is Aib (alpha-aminoisobutyric acid)
  MISC_FEATURE (14)..(14): Xaa is Nle (Norleucine)
  MISC_FEATURE (24)..(24): The epsilon amino group of Lys has:[(4S)-4-carboxy-4-[[(4S)-4-carboxy-4-[[(4S)-4-carboxy-4-(17-c arboxyheptadecanoylamino)butanoyl]amino]butanoyl]amino]butanoyl]-
  MISC_FEATURE (31)..(31): C-terminal amidation

SEQ ID NO: 63 - protein, 31 aa, ARTIFICIAL; identical to SEQ ID NO: 48
  Synthetic polypeptide
  MISC_FEATURE (1)..(1): Xaa is Tyr or d-Tyr
  MISC_FEATURE (2)..(2): Xaa is Ala or Aib (alpha-aminoisobutyric acid)
  MISC_FEATURE (14)..(14): Xaa is Asp, Leu, or Nle (norleucine)
  MISC_FEATURE (16)..(16): Xaa is Lys or Ala
  MISC_FEATURE (18)..(18): Xaa is His or Arg
  MISC_FEATURE (20)..(20): Xaa is Gln, Glu, or Aib (alpha-aminoisobutyric acid)
  MISC_FEATURE (24)..(24): Modifying group attached to epsilon amino group of lysine
  MISC_FEATURE (31)..(31): Xaa is Gly or Pro

SEQ ID NO: 64 - protein, 31 aa, ARTIFICIAL; identical to SEQ ID NO: 48
  Synthetic polypeptide
  MISC_FEATURE (1)..(1): Xaa is Tyr or d-Tyr
  MISC_FEATURE (2)..(2): Xaa is Ala, d-Ala, or Aib (alpha-aminoisobutyric acid)
  MISC_FEATURE (14)..(14): Xaa is Leu, Met, or Nle (norleucine)
  MISC_FEATURE (16)..(16): Xaa is Lys or Ala
  MISC_FEATURE (18)..(18): Xaa is Arg or His
  MISC_FEATURE (20)..(20): Xaa is Gln, Glu, or Aib (alpha-aminoisobutyric acid)
  MISC_FEATURE (24)..(24): Modifying group attached to epsilon amino group of lysine
  MISC_FEATURE (31)..(31): Xaa is Gly or Pro

SEQ ID NO: 65 - protein, 31 aa, ARTIFICIAL; identical to SEQ ID NO: 48
  Synthetic polypeptide
  MISC_FEATURE (1)..(1): Xaa is Tyr, Ac-Tyr, d-Tyr or Ac-d-Tyr
  MISC_FEATURE (2)..(2): Xaa is Ala, d-Ala, or Aib (alpha-aminoisobutyric acid)
  MISC_FEATURE (14)..(14): Xaa is Leu, Met, Asp or Nle (norleucine)
  MISC_FEATURE (16)..(16): Xaa is Lys or Ala
  MISC_FEATURE (18)..(18): Xaa is Arg or His
  MISC_FEATURE (20)..(20): Xaa is Gln, Glu, or Aib (alpha-aminoisobutyric acid)
  MISC_FEATURE (24)..(24): Modifying group attached to epsilon amino group of lysine
  MISC_FEATURE (31)..(31): Xaa is Gly or Pro